European Patent Application EP 4 786 575 A1, published August 5, 2026. Title: OLEAGINUS YEAST AND PRODUCTION OF MICROBIAL OILS. Applicant: IBERIA BIOENERGY. Application EP. The sequence listing filed with the application follows.

SEQUENCE LISTING (2 sequences)

SEQ ID NO: 1 - RNA, 613 nt, Rhodosporidium toruloides
  source 1..613: mol_type = rRNA
ttccgtagggtgaacctgcggaaggatcattagtgaatattagggtgtccaacttaacttggagcccgaccctcactttctaaccctgtgcatttgtcttgggtagtagcttgcgtcagcgagcgaatcccatttcacttacaaacacaaagtctatgaatgtaacaaatttataacaaaacaaaactttcaacaacggatctcttggctctcgcatcgatgaagaacgcagcgaaatgcgatacgtaatgtgaattgcagaattcagtgaatcatcgaatctttgaacgcaccttgcgctccatggtattccgtggagcatgcctgtttgagtgtcatgaattcttcaacccacctctttcttagtgaatcaggcggtgtttggattctgagcgctgctggcttcgcggcctagctcgctcgtaatgcattagcatccgcaatcaaacttcggattgactcggcgtaatagactattcgctgaggattctggtctctgactggagccgggtaaggttaaagggagctactaatcctcatgtctatcttgagattagacctcaaatcaggtaggactacccgctgaacttaagcatatcaatagccggaggaa

SEQ ID NO: 2 - RNA, 604 nt, Rhodosporidium toruloides
  source 1..604: mol_type = rRNA
gaacctgcggaaggatcattagtgaatattagggtgtccaacttaacttggagcccgaccctcactttctaaccctgtgcatttgtcttgggtagtagcttgcgtcagcgagcgaatcccatttcacttacaaacacaaagtctatgaatgtaacaaatttataacaaaacaaaactttcaacaacggatctcttggctctcgcatcgatgaagaacgcagcgaaatgcgatacgtaatgtgaattgcagaattcagtgaatcatcgaatctttgaacgcaccttgcgctccatggtattccgtggagcatgcctgtttgagtgtcatgaattcttcaacccacctctttcttagtgaatcaggcggtgtttggattctgagcgctgctggcttcgcggcctagctcgctcgtaatgcattagcatccgcaatcaaacttcggattgactcggcgtaatagactattcgctgaggattctggtctctgactggagccgggtaaggttaaagggagctactaatcctcatgtctatcttgagattagacctcaaatcaggtaggactacccgctgaacttaagcatatcaataagccgggaggaa